European Patent Specification EP 3 784 288 B1, published May 27, 2026. Title: Modified AAV capsid polypeptides for Treatment of Muscular Diseases. Applicant: Universität Heidelberg. The sequence listing filed with the application follows.

SEQUENCE LISTING (55 sequences)

SEQ ID NO: 1 - protein, 7 aa, Artificial
  consensus sequence of binding peptide
  misc_feature (4)..(7): X can be any amino acid
RGDXXXX

SEQ ID NO: 2 - protein, 7 aa, Artificial
  binding peptide P1
RGDLGLS

SEQ ID NO: 3 - protein, 7 aa, Artificial
  binding paptide P3
RGDAVGV

SEQ ID NO: 4 - protein, 8 aa, Artificial
  binding peptide A1
MPLGAAGA

SEQ ID NO: 5 - protein, 8 aa, Artificial
  binding peptide K3
RGDLRVSA

SEQ ID NO: 6 - protein, 7 aa, Artificial
  binding peptide MTP
ASSLNIA

SEQ ID NO: 7 - protein, 21 aa, Artificial
  AAV9_P1 insertion site
NHQGQSGRGDLGLSAQAAQTG

SEQ ID NO: 8 - protein, 21 aa, Artificial
  AAV9_P3 insertion site
NHQGQSGRGDAVGVAQAAQTG

SEQ ID NO: 9 - protein, 21 aa, Artificial
  AAVpo1_A1 insertion site
NNQGQRGMPLGAAGAQAATVG

SEQ ID NO: 10 - protein, 21 aa, Artificial
  AAV9_K3 insertion site
HQSGQAGRGDLRVSAQAATGW

SEQ ID NO: 11 - protein, 21 aa, Artificial
  AAV-MTP insertion site
NLQRGNTGASSLNIAGLSRQA

SEQ ID NO: 12 - protein, 745 aa, Artificial
  AAV9_P1 capsid polypeptide, insertion site 588
MAADGYLPDWLEDNLSEGIREWWALKPGAPQPKANQQHQDNARGLVLPGYKYLGPGNGLDKGEPVNAADAAALEHDKAYDQQLKAGDNPYLKYNHADAEFQERLKEDTSFGGNLGRAVFQAKKRLLEPLGLVEEAAKTAPGKKRPVEQSPQEPDSSAGIGKSGAQPAKKRLNFGQTGDTESVPDPQPIGEPPAAPSGVGSLTMASGGGAPVADNNEGADGVGSSSGNWHCDSQWLGDRVITTSTRTWALPTYNNHLYKQISNSTSGGSSNDNAYFGYSTPWGYFDFNRFHCHFSPRDWQRLINNNWGFRPKRLNFKLFNIQVKEVTDNNGVKTIANNLTSTVQVFTDSDYQLPYVLGSAHEGCLPPFPADVFMIPQYGYLTLNDGSQAVGRSSFYCLEYFPSQMLRTGNNFQFSYEFENVPFHSSYAHSQSLDRLMNPLIDQYLYYLSKTINGSGQNQQTLKFSVAGPSNMAVQGRNYIPGPSYRQQRVSTTVTQNNNSEFAWPGASSWALNGRNSLMNPGPAMASHKEGEDRFFPLSGSLIFGKQGTGRDNVDADKVMITNEEEIKTTNPVATESYGQVATNHQGQSGRGDLGLSAQAAQTGWVQNQGILPGMVWQDRDVYLQGPIWAKIPHTDGNFHPSPLMGGFGMKHPPPQILIKNTPVPADPPTAFNKDKLNSFITQYSTGQVSVEIEWELQKENSKRWNPEIQYTSNYYKSNNVEFAVNTEGVYSEPRPIGTRYLTRNL

SEQ ID NO: 13 - DNA, 2238 bp, Artificial
  AAV9_P1 capsid polypeptide encoding, insertion site amino acid 588
atggctgccgatggttatcttccagattggctcgaggacaaccttagtgaaggaattcgcgagtggtgggctttgaaacctggagcccctcaacccaaggcaaatcaacaacatcaagacaacgctcgaggtcttgtgcttccgggttacaaataccttggacccggcaacggactcgacaagggggagccggtcaacgcagcagacgcggcggccctcgagcacgacaaggcctacgaccagcagctcaaggccggagacaacccgtacctcaagtacaaccacgccgacgccgagttccaggagcggctcaaagaagatacgtcttttgggggcaacctcgggcgagcagtcttccaggccaaaaagaggcttcttgaacctcttggtctggttgaggaagcggctaagacggctcctggaaagaagaggcctgtagagcagtctcctcaggaaccggactcctccgcgggtattggcaaatcgggtgcacagcccgctaaaaagagactcaatttcggtcagactggcgacacagagtcagtcccagaccctcaaccaatcggagaacctcccgcagccccctcaggtgtgggatctcttacaatggcttcaggtggtggcgcaccagtggcagacaataacgaaggtgccgatggagtgggtagttcctcgggaaattggcattgcgattcccaatggctgggggacagagtcatcaccaccagcacccgaacctgggccctgcccacctacaacaatcacctctacaagcaaatctccaacagcacatctggaggatcttcaaatgacaacgcctacttcggctacagcaccccctgggggtattttgacttcaacagattccactgccacttctcaccacgtgactggcagcgactcatcaacaacaactggggattccggcctaagcgactcaacttcaagctcttcaacattcaggtcaaagaggttacggacaacaatggagtcaagaccatcgccaataaccttaccagcacggtccaggtcttcacggactcagactatcagctcccgtacgtgctcgggtcggctcacgagggctgcctcccgccgttcccagcggacgttttcatgattcctcagtacgggtatctgacgcttaatgatggaagccaggccgtgggtcgttcgtccttttactgcctggaatatttcccgtcgcaaatgctaagaacgggtaacaacttccagttcagctacgagtttgagaacgtacctttccatagcagctacgctcacagccaaagcctggaccgactaatgaatccactcatcgaccaatacttgtactatctctcaaagactattaacggttctggacagaatcaacaaacgctaaaattcagtgtggccggacccagcaacatggctgtccagggaagaaactacatacctggacccagctaccgacaacaacgtgtctcaaccactgtgactcaaaacaacaacagcgaatttgcttggcctggagcttcttcttgggctctcaatggacgtaatagcttgatgaatcctggacctgctatggccagccacaaagaaggagaggaccgtttctttcctttgtctggatctttaatttttggcaaacaaggaactggaagagacaacgtggatgcggacaaagtcatgataaccaacgaagaagaaattaaaactactaacccggtagcaacggagtcctatggacaagtggccacaaaccaccagggccagagtggccgcggcgatctgggcctgagcgcccaggcggcccagaccggctgggttcaaaaccaaggaatacttccgggtatggtttggcaggacagagatgtgtacctgcaaggacccatttgggccaaaattcctcacacggacggcaactttcacccttctccgctgatgggagggtttggaatgaaacacccgcctcctcagatcctcatcaaaaacacacctgtacctgcggatcctccaacggccttcaacaaggacaagctgaactctttcatcacccagtattctactggccaagtcagcgtggagatcgagtgggagctgcagaaggaaaacagcaagcgctggaacccggagatccagtacacttccaactattacaagtctaataatgttgaatttgctgttaatactgaaggtgtatatagtgaaccccgccccattggcaccagatacctgactcgtaatctgtaa

SEQ ID NO: 14 - protein, 745 aa, Artificial
  AAV9LD_P1 capsid polypeptide, insertion site 588
MAADGYLPDWLEDNLSEGIREWWALKPGAPQPKANQQHQDNARGLVLPGYKYLGPGNGLDKGEPVNAADAAALEHDKAYDQQLKAGDNPYLKYNHADAEFQERLKEDTSFGGNLGRAVFQAKKRLLEPLGLVEEAAKTAPGKKRPVEQSPQEPDSSAGIGKSGAQPAKKRLNFGQTGDTESVPDPQPIGEPPAAPSGVGSLTMASGGGAPVADNNEGADGVGSSSGNWHCDSQWLGDRVITTSTRTWALPTYNNHLYKQISNSTSGGSSNDNAYFGYSTPWGYFDFNRFHCHFSPRDWQRLINNNWGFRPKRLNFKLFNIQVKEVTDNNGVKTIANNLTSTVQVFTDSDYQLPYVLGSAHEGCLPPFPADVFMIPQYGYLTLNDGSQAVGRSSFYCLEYFPSQMLRTGNNFQFSYEFENVPFHSSYAHSQSLDRLMNPLIDQYLYYLSKTINGSGQNQQTLKFSVAGPSNMAVQGRNYIPGPSYRQQRVSTTVTQNNNSEFAWAAASSWALNGRNSLMNPGPAMASHKEGEDRFFPLSGSLIFGKQGTGRDNVDADKVMITNEEEIKTTNPVATESYGQVATNHQGQSGRGDLGLSAQAAQTGWVQNQGILPGMVWQDRDVYLQGPIWAKIPHTDGNFHPSPLMGGFGMKHPPPQILIKNTPVPADPPTAFNKDKLNSFITQYSTGQVSVEIEWELQKENSKRWNPEIQYTSNYYKSNNVEFAVNTEGVYSEPRPIGTRYLTRNL

SEQ ID NO: 15 - DNA, 2238 bp, Artificial
  AAV9LD_P1 capsid polypeptide encoding, insertion site amino acid 588
atggctgccgatggttatcttccagattggctcgaggacaaccttagtgaaggaattcgcgagtggtgggctttgaaacctggagcccctcaacccaaggcaaatcaacaacatcaagacaacgctcgaggtcttgtgcttccgggttacaaataccttggacccggcaacggactcgacaagggggagccggtcaacgcagcagacgcggcggccctcgagcacgacaaggcctacgaccagcagctcaaggccggagacaacccgtacctcaagtacaaccacgccgacgccgagttccaggagcggctcaaagaagatacgtcttttgggggcaacctcgggcgagcagtcttccaggccaaaaagaggcttcttgaacctcttggtctggttgaggaagcggctaagacggctcctggaaagaagaggcctgtagagcagtctcctcaggaaccggactcctccgcgggtattggcaaatcgggtgcacagcccgctaaaaagagactcaatttcggtcagactggcgacacagagtcagtcccagaccctcaaccaatcggagaacctcccgcagccccctcaggtgtgggatctcttacaatggcttcaggtggtggcgcaccagtggcagacaataacgaaggtgccgatggagtgggtagttcctcgggaaattggcattgcgattcccaatggctgggggacagagtcatcaccaccagcacccgaacctgggccctgcccacctacaacaatcacctctacaagcaaatctccaacagcacatctggaggatcttcaaatgacaacgcctacttcggctacagcaccccctgggggtattttgacttcaacagattccactgccacttctcaccacgtgactggcagcgactcatcaacaacaactggggattccggcctaagcgactcaacttcaagctcttcaacattcaggtcaaagaggttacggacaacaatggagtcaagaccatcgccaataaccttaccagcacggtccaggtcttcacggactcagactatcagctcccgtacgtgctcgggtcggctcacgagggctgcctcccgccgttcccagcggacgttttcatgattcctcagtacgggtatctgacgcttaatgatggaagccaggccgtgggtcgttcgtccttttactgcctggaatatttcccgtcgcaaatgctaagaacgggtaacaacttccagttcagctacgagtttgagaacgtacctttccatagcagctacgctcacagccaaagcctggaccgactaatgaatccactcatcgaccaatacttgtactatctctcaaagactattaacggttctggacagaatcaacaaacgctaaaattcagtgtggccggacccagcaacatggctgtccagggaagaaactacatacctggacccagctaccgacaacaacgtgtctcaaccactgtgactcaaaacaacaacagcgaatttgcttgggctgcagcttcttcttgggctctcaatggacgtaatagcttgatgaatcctggacctgctatggccagccacaaagaaggagaggaccgtttctttcctttgtctggatctttaatttttggcaaacaaggaactggaagagacaacgtggatgcggacaaagtcatgataaccaacgaagaagaaattaaaactactaacccggtagcaacggagtcctatggacaagtggccacaaaccaccagggccagagtggccgcggcgatctgggcctgagcgcccaggcggcccagaccggctgggttcaaaaccaaggaatacttccgggtatggtttggcaggacagagatgtgtacctgcaaggacccatttgggccaaaattcctcacacggacggcaactttcacccttctccgctgatgggagggtttggaatgaaacacccgcctcctcagatcctcatcaaaaacacacctgtacctgcggatcctccaacggccttcaacaaggacaagctgaactctttcatcacccagtattctactggccaagtcagcgtggagatcgagtgggagctgcagaaggaaaacagcaagcgctggaacccggagatccagtacacttccaactattacaagtctaataatgttgaatttgctgttaatactgaaggtgtatatagtgaaccccgccccattggcaccagatacctgactcgtaatctgtaa

SEQ ID NO: 16 - protein, 745 aa, Artificial
  AAV9_P1 capsid polypeptide, insertion site 589
MAADGYLPDWLEDNLSEGIREWWALKPGAPQPKANQQHQDNARGLVLPGYKYLGPGNGLDKGEPVNAADAAALEHDKAYDQQLKAGDNPYLKYNHADAEFQERLKEDTSFGGNLGRAVFQAKKRLLEPLGLVEEAAKTAPGKKRPVEQSPQEPDSSAGIGKSGAQPAKKRLNFGQTGDTESVPDPQPIGEPPAAPSGVGSLTMASGGGAPVADNNEGADGVGSSSGNWHCDSQWLGDRVITTSTRTWALPTYNNHLYKQISNSTSGGSSNDNAYFGYSTPWGYFDFNRFHCHFSPRDWQRLINNNWGFRPKRLNFKLFNIQVKEVTDNNGVKTIANNLTSTVQVFTDSDYQLPYVLGSAHEGCLPPFPADVFMIPQYGYLTLNDGSQAVGRSSFYCLEYFPSQMLRTGNNFQFSYEFENVPFHSSYAHSQSLDRLMNPLIDQYLYYLSKTINGSGQNQQTLKFSVAGPSNMAVQGRNYIPGPSYRQQRVSTTVTQNNNSEFAWPGASSWALNGRNSLMNPGPAMASHKEGEDRFFPLSGSLIFGKQGTGRDNVDADKVMITNEEEIKTTNPVATESYGQVATNHQSGQSGRGDLGLSAQAATGWVQNQGILPGMVWQDRDVYLQGPIWAKIPHTDGNFHPSPLMGGFGMKHPPPQILIKNTPVPADPPTAFNKDKLNSFITQYSTGQVSVEIEWELQKENSKRWNPEIQYTSNYYKSNNVEFAVNTEGVYSEPRPIGTRYLTRNL

SEQ ID NO: 17 - DNA, 2238 bp, Artificial
  AAV9_P1 capsid polypeptide 2 encoding, insertion site amino acid 589
atggctgccgatggttatcttccagattggctcgaggacaaccttagtgaaggaattcgcgagtggtgggctttgaaacctggagcccctcaacccaaggcaaatcaacaacatcaagacaacgctcgaggtcttgtgcttccgggttacaaataccttggacccggcaacggactcgacaagggggagccggtcaacgcagcagacgcggcggccctcgagcacgacaaggcctacgaccagcagctcaaggccggagacaacccgtacctcaagtacaaccacgccgacgccgagttccaggagcggctcaaagaagatacgtcttttgggggcaacctcgggcgagcagtcttccaggccaaaaagaggcttcttgaacctcttggtctggttgaggaagcggctaagacggctcctggaaagaagaggcctgtagagcagtctcctcaggaaccggactcctccgcgggtattggcaaatcgggtgcacagcccgctaaaaagagactcaatttcggtcagactggcgacacagagtcagtcccagaccctcaaccaatcggagaacctcccgcagccccctcaggtgtgggatctcttacaatggcttcaggtggtggcgcaccagtggcagacaataacgaaggtgccgatggagtgggtagttcctcgggaaattggcattgcgattcccaatggctgggggacagagtcatcaccaccagcacccgaacctgggccctgcccacctacaacaatcacctctacaagcaaatctccaacagcacatctggaggatcttcaaatgacaacgcctacttcggctacagcaccccctgggggtattttgacttcaacagattccactgccacttctcaccacgtgactggcagcgactcatcaacaacaactggggattccggcctaagcgactcaacttcaagctcttcaacattcaggtcaaagaggttacggacaacaatggagtcaagaccatcgccaataaccttaccagcacggtccaggtcttcacggactcagactatcagctcccgtacgtgctcgggtcggctcacgagggctgcctcccgccgttcccagcggacgttttcatgattcctcagtacgggtatctgacgcttaatgatggaagccaggccgtgggtcgttcgtccttttactgcctggaatatttcccgtcgcaaatgctaagaacgggtaacaacttccagttcagctacgagtttgagaacgtacctttccatagcagctacgctcacagccaaagcctggaccgactaatgaatccactcatcgaccaatacttgtactatctctcaaagactattaacggttctggacagaatcaacaaacgctaaaattcagtgtggccggacccagcaacatggctgtccagggaagaaactacatacctggacccagctaccgacaacaacgtgtctcaaccactgtgactcaaaacaacaacagcgaatttgcttggcctggagcttcttcttgggctctcaatggacgtaatagcttgatgaatcctggacctgctatggccagccacaaagaaggagaggaccgtttctttcctttgtctggatctttaatttttggcaaacaaggaactggaagagacaacgtggatgcggacaaagtcatgataaccaacgaagaagaaattaaaactactaacccggtagcaacggagtcctatggacaagtggccacaaaccaccagagtggccagagtggccgcggcgatctgggcctgagcgcccaggcggccaccggctgggttcaaaaccaaggaatacttccgggtatggtttggcaggacagagatgtgtacctgcaaggacccatttgggccaaaattcctcacacggacggcaactttcacccttctccgctgatgggagggtttggaatgaaacacccgcctcctcagatcctcatcaaaaacacacctgtacctgcggatcctccaacggccttcaacaaggacaagctgaactctttcatcacccagtattctactggccaagtcagcgtggagatcgagtgggagctgcagaaggaaaacagcaagcgctggaacccggagatccagtacacttccaactattacaagtctaataatgttgaatttgctgttaatactgaaggtgtatatagtgaaccccgccccattggcaccagatacctgactcgtaatctgtaa

SEQ ID NO: 18 - protein, 745 aa, Artificial
  AAV9_P3 capsid polypeptide, insertion site 588
MAADGYLPDWLEDNLSEGIREWWALKPGAPQPKANQQHQDNARGLVLPGYKYLGPGNGLDKGEPVNAADAAALEHDKAYDQQLKAGDNPYLKYNHADAEFQERLKEDTSFGGNLGRAVFQAKKRLLEPLGLVEEAAKTAPGKKRPVEQSPQEPDSSAGIGKSGAQPAKKRLNFGQTGDTESVPDPQPIGEPPAAPSGVGSLTMASGGGAPVADNNEGADGVGSSSGNWHCDSQWLGDRVITTSTRTWALPTYNNHLYKQISNSTSGGSSNDNAYFGYSTPWGYFDFNRFHCHFSPRDWQRLINNNWGFRPKRLNFKLFNIQVKEVTDNNGVKTIANNLTSTVQVFTDSDYQLPYVLGSAHEGCLPPFPADVFMIPQYGYLTLNDGSQAVGRSSFYCLEYFPSQMLRTGNNFQFSYEFENVPFHSSYAHSQSLDRLMNPLIDQYLYYLSKTINGSGQNQQTLKFSVAGPSNMAVQGRNYIPGPSYRQQRVSTTVTQNNNSEFAWPGASSWALNGRNSLMNPGPAMASHKEGEDRFFPLSGSLIFGKQGTGRDNVDADKVMITNEEEIKTTNPVATESYGQVATNHQGQSGRGDAVGVAQAAQTGWVQNQGILPGMVWQDRDVYLQGPIWAKIPHTDGNFHPSPLMGGFGMKHPPPQILIKNTPVPADPPTAFNKDKLNSFITQYSTGQVSVEIEWELQKENSKRWNPEIQYTSNYYKSNNVEFAVNTEGVYSEPRPIGTRYLTRNL

SEQ ID NO: 19 - DNA, 2238 bp, Artificial
  AAV9_P3 capsid polypeptide encoding, insertion site 588
atggctgccgatggttatcttccagattggctcgaggacaaccttagtgaaggaattcgcgagtggtgggctttgaaacctggagcccctcaacccaaggcaaatcaacaacatcaagacaacgctcgaggtcttgtgcttccgggttacaaataccttggacccggcaacggactcgacaagggggagccggtcaacgcagcagacgcggcggccctcgagcacgacaaggcctacgaccagcagctcaaggccggagacaacccgtacctcaagtacaaccacgccgacgccgagttccaggagcggctcaaagaagatacgtcttttgggggcaacctcgggcgagcagtcttccaggccaaaaagaggcttcttgaacctcttggtctggttgaggaagcggctaagacggctcctggaaagaagaggcctgtagagcagtctcctcaggaaccggactcctccgcgggtattggcaaatcgggtgcacagcccgctaaaaagagactcaatttcggtcagactggcgacacagagtcagtcccagaccctcaaccaatcggagaacctcccgcagccccctcaggtgtgggatctcttacaatggcttcaggtggtggcgcaccagtggcagacaataacgaaggtgccgatggagtgggtagttcctcgggaaattggcattgcgattcccaatggctgggggacagagtcatcaccaccagcacccgaacctgggccctgcccacctacaacaatcacctctacaagcaaatctccaacagcacatctggaggatcttcaaatgacaacgcctacttcggctacagcaccccctgggggtattttgacttcaacagattccactgccacttctcaccacgtgactggcagcgactcatcaacaacaactggggattccggcctaagcgactcaacttcaagctcttcaacattcaggtcaaagaggttacggacaacaatggagtcaagaccatcgccaataaccttaccagcacggtccaggtcttcacggactcagactatcagctcccgtacgtgctcgggtcggctcacgagggctgcctcccgccgttcccagcggacgttttcatgattcctcagtacgggtatctgacgcttaatgatggaagccaggccgtgggtcgttcgtccttttactgcctggaatatttcccgtcgcaaatgctaagaacgggtaacaacttccagttcagctacgagtttgagaacgtacctttccatagcagctacgctcacagccaaagcctggaccgactaatgaatccactcatcgaccaatacttgtactatctctcaaagactattaacggttctggacagaatcaacaaacgctaaaattcagtgtggccggacccagcaacatggctgtccagggaagaaactacatacctggacccagctaccgacaacaacgtgtctcaaccactgtgactcaaaacaacaacagcgaatttgcttggcctggagcttcttcttgggctctcaatggacgtaatagcttgatgaatcctggacctgctatggccagccacaaagaaggagaggaccgtttctttcctttgtctggatctttaatttttggcaaacaaggaactggaagagacaacgtggatgcggacaaagtcatgataaccaacgaagaagaaattaaaactactaacccggtagcaacggagtcctatggacaagtggccacaaaccaccagggccagagtggccgcggcgatgcggtgggcgtggcccaggcggcccagaccggctgggttcaaaaccaaggaatacttccgggtatggtttggcaggacagagatgtgtacctgcaaggacccatttgggccaaaattcctcacacggacggcaactttcacccttctccgctgatgggagggtttggaatgaaacacccgcctcctcagatcctcatcaaaaacacacctgtacctgcggatcctccaacggccttcaacaaggacaagctgaactctttcatcacccagtattctactggccaagtcagcgtggagatcgagtgggagctgcagaaggaaaacagcaagcgctggaacccggagatccagtacacttccaactattacaagtctaataatgttgaatttgctgttaatactgaaggtgtatatagtgaaccccgccccattggcaccagatacctgactcgtaatctgtaa

SEQ ID NO: 20 - protein, 745 aa, Artificial
  AAV9_P3 capsid polypeptide 2, insertion site 589
MAADGYLPDWLEDNLSEGIREWWALKPGAPQPKANQQHQDNARGLVLPGYKYLGPGNGLDKGEPVNAADAAALEHDKAYDQQLKAGDNPYLKYNHADAEFQERLKEDTSFGGNLGRAVFQAKKRLLEPLGLVEEAAKTAPGKKRPVEQSPQEPDSSAGIGKSGAQPAKKRLNFGQTGDTESVPDPQPIGEPPAAPSGVGSLTMASGGGAPVADNNEGADGVGSSSGNWHCDSQWLGDRVITTSTRTWALPTYNNHLYKQISNSTSGGSSNDNAYFGYSTPWGYFDFNRFHCHFSPRDWQRLINNNWGFRPKRLNFKLFNIQVKEVTDNNGVKTIANNLTSTVQVFTDSDYQLPYVLGSAHEGCLPPFPADVFMIPQYGYLTLNDGSQAVGRSSFYCLEYFPSQMLRTGNNFQFSYEFENVPFHSSYAHSQSLDRLMNPLIDQYLYYLSKTINGSGQNQQTLKFSVAGPSNMAVQGRNYIPGPSYRQQRVSTTVTQNNNSEFAWPGASSWALNGRNSLMNPGPAMASHKEGEDRFFPLSGSLIFGKQGTGRDNVDADKVMITNEEEIKTTNPVATESYGQVATNHQSGQSGRGDAVGVAQAATGWVQNQGILPGMVWQDRDVYLQGPIWAKIPHTDGNFHPSPLMGGFGMKHPPPQILIKNTPVPADPPTAFNKDKLNSFITQYSTGQVSVEIEWELQKENSKRWNPEIQYTSNYYKSNNVEFAVNTEGVYSEPRPIGTRYLTRNL

SEQ ID NO: 21 - DNA, 2238 bp, Artificial
  AAV9_P3 capsid polypeptide 2 encoding, insertion site 589
atggctgccgatggttatcttccagattggctcgaggacaaccttagtgaaggaattcgcgagtggtgggctttgaaacctggagcccctcaacccaaggcaaatcaacaacatcaagacaacgctcgaggtcttgtgcttccgggttacaaataccttggacccggcaacggactcgacaagggggagccggtcaacgcagcagacgcggcggccctcgagcacgacaaggcctacgaccagcagctcaaggccggagacaacccgtacctcaagtacaaccacgccgacgccgagttccaggagcggctcaaagaagatacgtcttttgggggcaacctcgggcgagcagtcttccaggccaaaaagaggcttcttgaacctcttggtctggttgaggaagcggctaagacggctcctggaaagaagaggcctgtagagcagtctcctcaggaaccggactcctccgcgggtattggcaaatcgggtgcacagcccgctaaaaagagactcaatttcggtcagactggcgacacagagtcagtcccagaccctcaaccaatcggagaacctcccgcagccccctcaggtgtgggatctcttacaatggcttcaggtggtggcgcaccagtggcagacaataacgaaggtgccgatggagtgggtagttcctcgggaaattggcattgcgattcccaatggctgggggacagagtcatcaccaccagcacccgaacctgggccctgcccacctacaacaatcacctctacaagcaaatctccaacagcacatctggaggatcttcaaatgacaacgcctacttcggctacagcaccccctgggggtattttgacttcaacagattccactgccacttctcaccacgtgactggcagcgactcatcaacaacaactggggattccggcctaagcgactcaacttcaagctcttcaacattcaggtcaaagaggttacggacaacaatggagtcaagaccatcgccaataaccttaccagcacggtccaggtcttcacggactcagactatcagctcccgtacgtgctcgggtcggctcacgagggctgcctcccgccgttcccagcggacgttttcatgattcctcagtacgggtatctgacgcttaatgatggaagccaggccgtgggtcgttcgtccttttactgcctggaatatttcccgtcgcaaatgctaagaacgggtaacaacttccagttcagctacgagtttgagaacgtacctttccatagcagctacgctcacagccaaagcctggaccgactaatgaatccactcatcgaccaatacttgtactatctctcaaagactattaacggttctggacagaatcaacaaacgctaaaattcagtgtggccggacccagcaacatggctgtccagggaagaaactacatacctggacccagctaccgacaacaacgtgtctcaaccactgtgactcaaaacaacaacagcgaatttgcttggcctggagcttcttcttgggctctcaatggacgtaatagcttgatgaatcctggacctgctatggccagccacaaagaaggagaggaccgtttctttcctttgtctggatctttaatttttggcaaacaaggaactggaagagacaacgtggatgcggacaaagtcatgataaccaacgaagaagaaattaaaactactaacccggtagcaacggagtcctatggacaagtggccacaaaccaccagagtggccagagtggccgcggcgatgcggtgggcgtggcccaggcggccaccggctgggttcaaaaccaaggaatacttccgggtatggtttggcaggacagagatgtgtacctgcaaggacccatttgggccaaaattcctcacacggacggcaactttcacccttctccgctgatgggagggtttggaatgaaacacccgcctcctcagatcctcatcaaaaacacacctgtacctgcggatcctccaacggccttcaacaaggacaagctgaactctttcatcacccagtattctactggccaagtcagcgtggagatcgagtgggagctgcagaaggaaaacagcaagcgctggaacccggagatccagtacacttccaactattacaagtctaataatgttgaatttgctgttaatactgaaggtgtatatagtgaaccccgccccattggcaccagatacctgactcgtaatctgtaa

SEQ ID NO: 22 - protein, 745 aa, Artificial
  AAV9LD_P1 capsid polypeptide 2, insertion site 589
MAADGYLPDWLEDNLSEGIREWWALKPGAPQPKANQQHQDNARGLVLPGYKYLGPGNGLDKGEPVNAADAAALEHDKAYDQQLKAGDNPYLKYNHADAEFQERLKEDTSFGGNLGRAVFQAKKRLLEPLGLVEEAAKTAPGKKRPVEQSPQEPDSSAGIGKSGAQPAKKRLNFGQTGDTESVPDPQPIGEPPAAPSGVGSLTMASGGGAPVADNNEGADGVGSSSGNWHCDSQWLGDRVITTSTRTWALPTYNNHLYKQISNSTSGGSSNDNAYFGYSTPWGYFDFNRFHCHFSPRDWQRLINNNWGFRPKRLNFKLFNIQVKEVTDNNGVKTIANNLTSTVQVFTDSDYQLPYVLGSAHEGCLPPFPADVFMIPQYGYLTLNDGSQAVGRSSFYCLEYFPSQMLRTGNNFQFSYEFENVPFHSSYAHSQSLDRLMNPLIDQYLYYLSKTINGSGQNQQTLKFSVAGPSNMAVQGRNYIPGPSYRQQRVSTTVTQNNNSEFAWAAASSWALNGRNSLMNPGPAMASHKEGEDRFFPLSGSLIFGKQGTGRDNVDADKVMITNEEEIKTTNPVATESYGQVATNHQSGQSGRGDLGLSAQAATGWVQNQGILPGMVWQDRDVYLQGPIWAKIPHTDGNFHPSPLMGGFGMKHPPPQILIKNTPVPADPPTAFNKDKLNSFITQYSTGQVSVEIEWELQKENSKRWNPEIQYTSNYYKSNNVEFAVNTEGVYSEPRPIGTRYLTRNL

SEQ ID NO: 23 - DNA, 2238 bp, Artificial
  AAV9LD_P1 capsid polypeptide 2 encoding, insertion site amno acid 589
atggctgccgatggttatcttccagattggctcgaggacaaccttagtgaaggaattcgcgagtggtgggctttgaaacctggagcccctcaacccaaggcaaatcaacaacatcaagacaacgctcgaggtcttgtgcttccgggttacaaataccttggacccggcaacggactcgacaagggggagccggtcaacgcagcagacgcggcggccctcgagcacgacaaggcctacgaccagcagctcaaggccggagacaacccgtacctcaagtacaaccacgccgacgccgagttccaggagcggctcaaagaagatacgtcttttgggggcaacctcgggcgagcagtcttccaggccaaaaagaggcttcttgaacctcttggtctggttgaggaagcggctaagacggctcctggaaagaagaggcctgtagagcagtctcctcaggaaccggactcctccgcgggtattggcaaatcgggtgcacagcccgctaaaaagagactcaatttcggtcagactggcgacacagagtcagtcccagaccctcaaccaatcggagaacctcccgcagccccctcaggtgtgggatctcttacaatggcttcaggtggtggcgcaccagtggcagacaataacgaaggtgccgatggagtgggtagttcctcgggaaattggcattgcgattcccaatggctgggggacagagtcatcaccaccagcacccgaacctgggccctgcccacctacaacaatcacctctacaagcaaatctccaacagcacatctggaggatcttcaaatgacaacgcctacttcggctacagcaccccctgggggtattttgacttcaacagattccactgccacttctcaccacgtgactggcagcgactcatcaacaacaactggggattccggcctaagcgactcaacttcaagctcttcaacattcaggtcaaagaggttacggacaacaatggagtcaagaccatcgccaataaccttaccagcacggtccaggtcttcacggactcagactatcagctcccgtacgtgctcgggtcggctcacgagggctgcctcccgccgttcccagcggacgttttcatgattcctcagtacgggtatctgacgcttaatgatggaagccaggccgtgggtcgttcgtccttttactgcctggaatatttcccgtcgcaaatgctaagaacgggtaacaacttccagttcagctacgagtttgagaacgtacctttccatagcagctacgctcacagccaaagcctggaccgactaatgaatccactcatcgaccaatacttgtactatctctcaaagactattaacggttctggacagaatcaacaaacgctaaaattcagtgtggccggacccagcaacatggctgtccagggaagaaactacatacctggacccagctaccgacaacaacgtgtctcaaccactgtgactcaaaacaacaacagcgaatttgcttgggctgcagcttcttcttgggctctcaatggacgtaatagcttgatgaatcctggacctgctatggccagccacaaagaaggagaggaccgtttctttcctttgtctggatctttaatttttggcaaacaaggaactggaagagacaacgtggatgcggacaaagtcatgataaccaacgaagaagaaattaaaactactaacccggtagcaacggagtcctatggacaagtggccacaaaccaccagagtggccagagtggccgcggcgatctgggcctgagcgcccaggcggccaccggctgggttcaaaaccaaggaatacttccgggtatggtttggcaggacagagatgtgtacctgcaaggacccatttgggccaaaattcctcacacggacggcaactttcacccttctccgctgatgggagggtttggaatgaaacacccgcctcctcagatcctcatcaaaaacacacctgtacctgcggatcctccaacggccttcaacaaggacaagctgaactctttcatcacccagtattctactggccaagtcagcgtggagatcgagtgggagctgcagaaggaaaacagcaagcgctggaacccggagatccagtacacttccaactattacaagtctaataatgttgaatttgctgttaatactgaaggtgtatatagtgaaccccgccccattggcaccagatacctgactcgtaatctgtaa

SEQ ID NO: 24 - protein, 745 aa, Artificial
  AAV9LD_P3 capsid polypeptide, insertion site 588
MAADGYLPDWLEDNLSEGIREWWALKPGAPQPKANQQHQDNARGLVLPGYKYLGPGNGLDKGEPVNAADAAALEHDKAYDQQLKAGDNPYLKYNHADAEFQERLKEDTSFGGNLGRAVFQAKKRLLEPLGLVEEAAKTAPGKKRPVEQSPQEPDSSAGIGKSGAQPAKKRLNFGQTGDTESVPDPQPIGEPPAAPSGVGSLTMASGGGAPVADNNEGADGVGSSSGNWHCDSQWLGDRVITTSTRTWALPTYNNHLYKQISNSTSGGSSNDNAYFGYSTPWGYFDFNRFHCHFSPRDWQRLINNNWGFRPKRLNFKLFNIQVKEVTDNNGVKTIANNLTSTVQVFTDSDYQLPYVLGSAHEGCLPPFPADVFMIPQYGYLTLNDGSQAVGRSSFYCLEYFPSQMLRTGNNFQFSYEFENVPFHSSYAHSQSLDRLMNPLIDQYLYYLSKTINGSGQNQQTLKFSVAGPSNMAVQGRNYIPGPSYRQQRVSTTVTQNNNSEFAWAAASSWALNGRNSLMNPGPAMASHKEGEDRFFPLSGSLIFGKQGTGRDNVDADKVMITNEEEIKTTNPVATESYGQVATNHQGQSGRGDAVGVAQAAQTGWVQNQGILPGMVWQDRDVYLQGPIWAKIPHTDGNFHPSPLMGGFGMKHPPPQILIKNTPVPADPPTAFNKDKLNSFITQYSTGQVSVEIEWELQKENSKRWNPEIQYTSNYYKSNNVEFAVNTEGVYSEPRPIGTRYLTRNL

SEQ ID NO: 25 - DNA, 2238 bp, Artificial
  AAV9LD_P3 capsid polypeptide encoding, insertion site amino acid 588
atggctgccgatggttatcttccagattggctcgaggacaaccttagtgaaggaattcgcgagtggtgggctttgaaacctggagcccctcaacccaaggcaaatcaacaacatcaagacaacgctcgaggtcttgtgcttccgggttacaaataccttggacccggcaacggactcgacaagggggagccggtcaacgcagcagacgcggcggccctcgagcacgacaaggcctacgaccagcagctcaaggccggagacaacccgtacctcaagtacaaccacgccgacgccgagttccaggagcggctcaaagaagatacgtcttttgggggcaacctcgggcgagcagtcttccaggccaaaaagaggcttcttgaacctcttggtctggttgaggaagcggctaagacggctcctggaaagaagaggcctgtagagcagtctcctcaggaaccggactcctccgcgggtattggcaaatcgggtgcacagcccgctaaaaagagactcaatttcggtcagactggcgacacagagtcagtcccagaccctcaaccaatcggagaacctcccgcagccccctcaggtgtgggatctcttacaatggcttcaggtggtggcgcaccagtggcagacaataacgaaggtgccgatggagtgggtagttcctcgggaaattggcattgcgattcccaatggctgggggacagagtcatcaccaccagcacccgaacctgggccctgcccacctacaacaatcacctctacaagcaaatctccaacagcacatctggaggatcttcaaatgacaacgcctacttcggctacagcaccccctgggggtattttgacttcaacagattccactgccacttctcaccacgtgactggcagcgactcatcaacaacaactggggattccggcctaagcgactcaacttcaagctcttcaacattcaggtcaaagaggttacggacaacaatggagtcaagaccatcgccaataaccttaccagcacggtccaggtcttcacggactcagactatcagctcccgtacgtgctcgggtcggctcacgagggctgcctcccgccgttcccagcggacgttttcatgattcctcagtacgggtatctgacgcttaatgatggaagccaggccgtgggtcgttcgtccttttactgcctggaatatttcccgtcgcaaatgctaagaacgggtaacaacttccagttcagctacgagtttgagaacgtacctttccatagcagctacgctcacagccaaagcctggaccgactaatgaatccactcatcgaccaatacttgtactatctctcaaagactattaacggttctggacagaatcaacaaacgctaaaattcagtgtggccggacccagcaacatggctgtccagggaagaaactacatacctggacccagctaccgacaacaacgtgtctcaaccactgtgactcaaaacaacaacagcgaatttgcttgggctgcagcttcttcttgggctctcaatggacgtaatagcttgatgaatcctggacctgctatggccagccacaaagaaggagaggaccgtttctttcctttgtctggatctttaatttttggcaaacaaggaactggaagagacaacgtggatgcggacaaagtcatgataaccaacgaagaagaaattaaaactactaacccggtagcaacggagtcctatggacaagtggccacaaaccaccagggccagagtggccgcggcgatgcggtgggcgtggcccaggcggcccagaccggctgggttcaaaaccaaggaatacttccgggtatggtttggcaggacagagatgtgtacctgcaaggacccatttgggccaaaattcctcacacggacggcaactttcacccttctccgctgatgggagggtttggaatgaaacacccgcctcctcagatcctcatcaaaaacacacctgtacctgcggatcctccaacggccttcaacaaggacaagctgaactctttcatcacccagtattctactggccaagtcagcgtggagatcgagtgggagctgcagaaggaaaacagcaagcgctggaacccggagatccagtacacttccaactattacaagtctaataatgttgaatttgctgttaatactgaaggtgtatatagtgaaccccgccccattggcaccagatacctgactcgtaatctgtaa

SEQ ID NO: 26 - protein, 745 aa, Artificial
  AAV9LD_P3 capsid polypeptide 2, insertion site 589
MAADGYLPDWLEDNLSEGIREWWALKPGAPQPKANQQHQDNARGLVLPGYKYLGPGNGLDKGEPVNAADAAALEHDKAYDQQLKAGDNPYLKYNHADAEFQERLKEDTSFGGNLGRAVFQAKKRLLEPLGLVEEAAKTAPGKKRPVEQSPQEPDSSAGIGKSGAQPAKKRLNFGQTGDTESVPDPQPIGEPPAAPSGVGSLTMASGGGAPVADNNEGADGVGSSSGNWHCDSQWLGDRVITTSTRTWALPTYNNHLYKQISNSTSGGSSNDNAYFGYSTPWGYFDFNRFHCHFSPRDWQRLINNNWGFRPKRLNFKLFNIQVKEVTDNNGVKTIANNLTSTVQVFTDSDYQLPYVLGSAHEGCLPPFPADVFMIPQYGYLTLNDGSQAVGRSSFYCLEYFPSQMLRTGNNFQFSYEFENVPFHSSYAHSQSLDRLMNPLIDQYLYYLSKTINGSGQNQQTLKFSVAGPSNMAVQGRNYIPGPSYRQQRVSTTVTQNNNSEFAWAAASSWALNGRNSLMNPGPAMASHKEGEDRFFPLSGSLIFGKQGTGRDNVDADKVMITNEEEIKTTNPVATESYGQVATNHQSGQSGRGDAVGVAQAATGWVQNQGILPGMVWQDRDVYLQGPIWAKIPHTDGNFHPSPLMGGFGMKHPPPQILIKNTPVPADPPTAFNKDKLNSFITQYSTGQVSVEIEWELQKENSKRWNPEIQYTSNYYKSNNVEFAVNTEGVYSEPRPIGTRYLTRNL

SEQ ID NO: 27 - DNA, 2238 bp, Artificial
  AAV9LD_P3 capsid polypeptide 2 encoding, insertion site amino acid 589
atggctgccgatggttatcttccagattggctcgaggacaaccttagtgaaggaattcgcgagtggtgggctttgaaacctggagcccctcaacccaaggcaaatcaacaacatcaagacaacgctcgaggtcttgtgcttccgggttacaaataccttggacccggcaacggactcgacaagggggagccggtcaacgcagcagacgcggcggccctcgagcacgacaaggcctacgaccagcagctcaaggccggagacaacccgtacctcaagtacaaccacgccgacgccgagttccaggagcggctcaaagaagatacgtcttttgggggcaacctcgggcgagcagtcttccaggccaaaaagaggcttcttgaacctcttggtctggttgaggaagcggctaagacggctcctggaaagaagaggcctgtagagcagtctcctcaggaaccggactcctccgcgggtattggcaaatcgggtgcacagcccgctaaaaagagactcaatttcggtcagactggcgacacagagtcagtcccagaccctcaaccaatcggagaacctcccgcagccccctcaggtgtgggatctcttacaatggcttcaggtggtggcgcaccagtggcagacaataacgaaggtgccgatggagtgggtagttcctcgggaaattggcattgcgattcccaatggctgggggacagagtcatcaccaccagcacccgaacctgggccctgcccacctacaacaatcacctctacaagcaaatctccaacagcacatctggaggatcttcaaatgacaacgcctacttcggctacagcaccccctgggggtattttgacttcaacagattccactgccacttctcaccacgtgactggcagcgactcatcaacaacaactggggattccggcctaagcgactcaacttcaagctcttcaacattcaggtcaaagaggttacggacaacaatggagtcaagaccatcgccaataaccttaccagcacggtccaggtcttcacggactcagactatcagctcccgtacgtgctcgggtcggctcacgagggctgcctcccgccgttcccagcggacgttttcatgattcctcagtacgggtatctgacgcttaatgatggaagccaggccgtgggtcgttcgtccttttactgcctggaatatttcccgtcgcaaatgctaagaacgggtaacaacttccagttcagctacgagtttgagaacgtacctttccatagcagctacgctcacagccaaagcctggaccgactaatgaatccactcatcgaccaatacttgtactatctctcaaagactattaacggttctggacagaatcaacaaacgctaaaattcagtgtggccggacccagcaacatggctgtccagggaagaaactacatacctggacccagctaccgacaacaacgtgtctcaaccactgtgactcaaaacaacaacagcgaatttgcttgggctgcagcttcttcttgggctctcaatggacgtaatagcttgatgaatcctggacctgctatggccagccacaaagaaggagaggaccgtttctttcctttgtctggatctttaatttttggcaaacaaggaactggaagagacaacgtggatgcggacaaagtcatgataaccaacgaagaagaaattaaaactactaacccggtagcaacggagtcctatggacaagtggccacaaaccaccagagtggccagagtggccgcggcgatgcggtgggcgtggcccaggcggccaccggctgggttcaaaaccaaggaatacttccgggtatggtttggcaggacagagatgtgtacctgcaaggacccatttgggccaaaattcctcacacggacggcaactttcacccttctccgctgatgggagggtttggaatgaaacacccgcctcctcagatcctcatcaaaaacacacctgtacctgcggatcctccaacggccttcaacaaggacaagctgaactctttcatcacccagtattctactggccaagtcagcgtggagatcgagtgggagctgcagaaggaaaacagcaagcgctggaacccggagatccagtacacttccaactattacaagtctaataatgttgaatttgctgttaatactgaaggtgtatatagtgaaccccgccccattggcaccagatacctgactcgtaatctgtaa

SEQ ID NO: 28 - protein, 744 aa, Artificial
  AAVS10_P1 capsid polypeptide
MAADGYLPDWLEDNLSEGIREWWALKPGAPKPKANQQKQDDGRGLVLPGYKYLGPFNGLDKGEPVNAADAAALEHDKAYDQQLQAGDNPYLRYNHADAEFQERLQEDTSFGGNLGRAVFQAKKRLLEPLGLVEEAAKTAPGKKRPVEQSPQEPDSSAGIGKSGAQPAKKRLNFGQTGDTESVPDPQPIGEPPAAPSGVGSLTMASGGGAPVADNNEGADGVGNASGNWHCDSQWLGDRVITTSTRTWALPTYNNHLYKQISSASTGATNDNTYFGYSTPWGYFDFNRFHCHFSPRDWQRLINNNWGFRPKRLNFKLFNIQVKEVTDNNGVKTIANNLTSTVQVFTDSDYQLPYVLGSAHEGCLPPFPADVFMIPQYGYLTLNDGSQAVGRSSFYCLEYFPSQMLRTGNNFQFSYEFENVPFHSSYAHSQSLDRLMNPLIDQYLYYLSKTINGSGQNQQTLKFSVAGPSNMAVQGRNYIPGPSYRQQRVSTTVTQNNNSEFAWPGASSWALNGRNSLMNPGPAMASHKEGEDRFFPLSGSLIFGKQGTGRDNVDADKVMITNEEEIKTTNPVATESYGQVATNHQGQSGRGDLGLSAQAAQTGWVQNQGILPGMVWQDRDVYLQGPIWAKIPHTDGNFHPSPLMGGFGMKHPPPQILIKNTPVPADPPTAFNKDKLNSFITQYSTGQVSVEIEWELQKENSKRWNPEIQYTSNYYKSNNVEFAVNTEGVYSEPRPIGTRYLTRNL

SEQ ID NO: 29 - DNA, 2235 bp, Artificial
  AAVS10_P1 capsid polypeptide encoding
atggctgccgatggttatcttccagattggctcgaggacaacctctctgagggcattcgcgagtggtgggctttgaaacctggagccccgaagcccaaagccaaccagcaaaagcaggacgacggccggggtctggtgcttcctggctacaagtacctcggacccttcaacggactcgacaagggggagcccgtcaacgcggcggacgcagcggccctcgagcacgacaaggcctacgaccagcagctgcaggcgggtgacaatccgtacctgcggtataaccacgccgacgccgagtttcaggagcgtctgcaagaagatacgtcttttgggggcaacctcgggcgagcagtcttccaggccaaaaagaggcttcttgaacctcttggtctggttgaggaagcggctaagacggctcctggaaagaaacgtccggtagagcagtcgccacaagagccagactcctccgcgggtattggcaaatcgggtgcacagcccgctaaaaagagactcaatttcggtcagactggcgacacagagtcagtcccagaccctcaaccaatcggagaacctcccgcagccccctcaggtgtgggatctcttacaatggcttcaggtggtggcgcaccagtggcagacaataacgaaggcgccgacggagtgggtaatgcctcgggaaattggcattgcgattcccaatggctgggggacagagtcatcaccaccagcacccgaacctgggccctgcccacctacaacaatcacctctacaagcaaatctccagtgcttcaacgggggccaccaacgacaacacctacttcggctacagcaccccctgggggtattttgacttcaacagattccactgccacttctcaccacgtgactggcagcgactcatcaacaacaactggggattccggcctaagcgactcaacttcaagctcttcaacattcaggtcaaagaggttacggacaacaatggagtcaagaccatcgccaataaccttaccagcacggtccaggtcttcacggactcagactatcagctcccgtacgtgctcgggtcggctcacgagggctgcctcccgccgttcccagcggacgttttcatgattcctcagtacgggtatctgacgcttaatgatggaagccaggccgtgggtcgttcgtccttttactgcctggaatatttcccgtcgcaaatgctaagaacgggtaacaacttccagttcagctacgagtttgagaacgtacctttccatagcagctacgctcacagccaaagcctggaccgactaatgaatccactcatcgaccaatacttgtactatctctcaaagactattaacggttctggacagaatcaacaaacgctaaaattcagtgtggccggacccagcaacatggctgtccagggaagaaactacatacctggacccagctaccgacaacaacgtgtctcaaccactgtgactcaaaacaacaacagcgaatttgcttggcctggagcttcttcttgggctctcaatggacgtaatagcttgatgaatcctggacctgctatggccagccacaaagaaggagaggaccgtttctttcctttgtctggatctttaatttttggcaaacaaggaactggaagagacaacgtggatgcggacaaagtcatgataaccaacgaagaagaaattaaaactactaacccggtagcaacggagtcctatggacaagtggccacaaaccaccagggccagagtggccgcggcgatctgggcctgagcgcccaggcggcccagaccggctgggttcaaaaccaaggaatacttccgggtatggtttggcaggacagagatgtgtacctgcaaggacccatttgggccaaaattcctcacacggacggcaactttcacccttctccgctgatgggagggtttggaatgaaacacccgcctcctcagatcctcatcaaaaacacacctgtacctgcggatcctccaacggccttcaacaaggacaagctgaactctttcatcacccagtattctactggccaagtcagcgtggagatcgagtgggagctgcagaaggaaaacagcaagcgctggaacccggagatccagtacacttccaactattacaagtctaataatgttgaatttgctgttaatactgaaggtgtatatagtgaaccccgccccattggcaccagatacctgactcgtaatctgtaa

SEQ ID NO: 30 - protein, 746 aa, Artificial
  AAVS1_P1 capsid polypeptide
MAADGYLPDWLEDNLSEGIREWWALKPGAPQPKANQQHQDNARGLVLPGYKYLGPGNGLDKGEPVNAADAAALEHDKAYDQQLKAGDNPYLRYNHADAEFQERLQEDTSFGGNLGRAVFQAKKRVLEPLGLVEEGAKTAPGKKRPVEPSPQRSPDSSTGIGKTGQQPAKKRLNFGQTGDTESVPDPQPIGEPPAAPAAVGPTTMASGGGAPMADNNEGADGVGNASGNWHCDSTWLGDRVITTSTRTWALPTYNNHLYKQISNGTSGGATNDNTYFGYSTPWGYFDFNRFHCHFSPRDWQRLINNNWGFRPKRLNFKLFNIQVKEVTDNNGVKTIANNLTSTVQVFTDSDYQLPYVLGSAHEGCLPPFPADVFMIPQYGYLTLNDGSQAVGRSSFYCLEYFPSQMLRTGNNFQFSYEFENVPFHSSYAHSQSLDRLMNPLIDQYLYYLSKTINGSGQNQQTLKFSVAGPSNMAVQGRNYIPGPSYRQQRVSTTVTQNNNSEFAWPGASSWALNGRNSLMNPGPAMASHKEGEDRFFPLSGSLIFGKQGTGRDNVDADKVMITNEEEIKTTNPVATESYGQVATNHQGQSGRGDLGLSAQAAQTGWVQNQGILPGMVWQDRDVYLQGPIWAKIPHTDGNFHPSPLMGGFGMKHPPPQILIKNTPVPADPPTAFNKDKLNSFITQYSTGQVSVEIEWELQKENSKRWNPEIQYTSNYYKSNNVEFAVNTEGVYSEPRPIGTRYLTRNL

SEQ ID NO: 31 - DNA, 2241 bp, Artificial
  AAVS1_P1 capsid polypeptide encoding
atggctgccgatggttatcttccagattggctcgaggacaaccttagtgaaggaattcgcgagtggtgggctttgaaacctggagcccctcaacccaaggcaaatcaacaacatcaagacaacgctcgaggtcttgtgcttccgggttacaaataccttggacccggcaacggactcgacaagggggagccggtcaacgcagcagacgcggcggccctcgagcacgacaaggcctacgaccagcagctcaaagcgggtgacaatccgtacctgcggtataaccacgccgacgccgagtttcaggagcgtctgcaagaagatacgtcttttgggggcaacctcgggcgagcagtcttccaggccaagaagcgggttctcgaacctctcggtctggttgaggaaggcgctaagacggctcctggaaagaaacgtccggtagagccatcaccccagcgttctccagactcctctacgggcatcggcaagacaggccagcagcccgctaaaaagagactcaatttcggtcagactggcgacacagagtcagtcccagaccctcaaccaatcggagaacctcccgcagcccccgctgctgtgggacctactacaatggcttcaggcggtggcgcaccaatggcagacaataacgaaggcgccgacggagtgggtaatgcctcaggaaattggcattgcgattccacatggctgggcgacagagtcatcaccaccagcacccgaacctgggccctgcccacctacaacaaccacctctacaagcaaatctccaacgggacatcgggaggagccaccaacgacaacacctacttcggctacagcaccccctgggggtattttgatttcaacagattccactgccatttctcaccacgtgactggcagcgactcatcaacaacaattggggattccggcccaagagactcaacttcaagctcttcaacattcaggtcaaagaggttacggacaacaatggagtcaagaccatcgccaataaccttaccagcacggtccaggtcttcacggactcagactatcagctcccgtacgtgctcgggtcggctcacgagggctgcctcccgccgttcccagcggacgttttcatgattcctcagtacgggtatctgacgcttaatgatggaagccaggccgtgggtcgttcgtccttttactgcctggaatatttcccgtcgcaaatgctaagaacgggtaacaacttccagttcagctacgagtttgagaacgtacctttccatagcagctacgctcacagccaaagcctggaccgactaatgaatccactcatcgaccaatacttgtactatctctcaaagactattaacggttctggacagaatcaacaaacgctaaaattcagtgtggccggacccagcaacatggctgtccagggaagaaactacatacctggacccagctaccgacaacaacgtgtctcaaccactgtgactcaaaacaacaacagcgaatttgcttggcctggagcttcttcttgggctctcaatggacgtaatagcttgatgaatcctggacctgctatggccagccacaaagaaggagaggaccgtttctttcctttgtctggatctttaatttttggcaaacaaggaactggaagagacaacgtggatgcggacaaagtcatgataaccaacgaagaagaaattaaaactactaacccggtagcaacggagtcctatggacaagtggccacaaaccaccagggccagagtggccgcggcgatctgggcctgagcgcccaggcggcccagaccggctgggttcaaaaccaaggaatacttccgggtatggtttggcaggacagagatgtgtacctgcaaggacccatttgggccaaaattcctcacacggacggcaactttcacccttctccgctgatgggagggtttggaatgaaacacccgcctcctcagatcctcatcaaaaacacacctgtacctgcggatcctccaacggccttcaacaaggacaagctgaactctttcatcacccagtattctactggccaagtcagcgtggagatcgagtgggagctgcagaaggaaaacagcaagcgctggaacccggagatccagtacacttccaactattacaagtctaataatgttgaatttgctgttaatactgaaggtgtatatagtgaaccccgccccattggcaccagatacctgactcgtaatctgtaa

SEQ ID NO: 32 - protein, 745 aa, Artificial
  AAVD20_P1 capsid polypeptide
MAADGYLPDWLEDNLSEGIREWWALKPGAPQPKANQQHQDNARGLVLPGYKYLGPGNGLDKGEPVNAADAAALEHDKAYDQQLKAGDNPYLKYNHADAEFQERLKEDTSFGGNLGRAVFQTKKRVLEPFGLVEEGAKTAPGKKRPVEQSPQEPDSSSGIVKTGQQPAKKRLNFGQTGDTESVPDPQPLGEPPATPSGVGSLTMASGGGAPMADNNEGADGVGNASGNWHCDSTWLGDRVITTSTRTWALPTYNNHLYKQISNGTSGGATNDNAYFGYSTPWGYFDFNRFHCHFSPRDWQRLINNNWGFRPKRLNFKLFNIQVKEVTDNNGVKTIANNLTSTVQVFTDSDYQLPYVLGSAHEGCLPPFPADVFMIPQYGYLTLNDGSQAVGRSSFYCLEYFPSQMLRTGNNFQFSYEFENVPFHSSYAHSQSLDRLMNPLIDQYLYYLSKTINGSGQNQQTLKFSVAGPSNMAVQGRNYIPGPSYRQQRVSTTVTQNNNSEFAWPGASSWALNGRNSLMNPGPAMASHKEGEDRFFPLSGSLIFGKQGTGRDNVDADKVMITNEEEIKTTNPVATESYGQVATNHQGQSGRGDLGLSAQAAQTGWVQNQGILPGMVWQDRDVYLQGPIWAKIPHTDGNFHPSPLMGGFGMKHPPPQILIKNTPVPADPPTAFNKDKLNSFITQYSTGQVSVEIEWELQKENSKRWNPEIQYTSNYYKSNNVEFAVNTEGVYSEPRPIGTRYLTRNL

SEQ ID NO: 33 - DNA, 2238 bp, Artificial
  AAVD20_P1 capsid polypeptide encoding
atggctgccgatggttatcttccagattggctcgaggacaaccttagtgaaggaattcgcgagtggtgggctttgaaacctggagcccctcaacccaaggcaaatcaacaacatcaagacaacgctcgaggtcttgtgcttccgggttacaaataccttggacccggcaacggactcgacaagggggagccggtcaacgcagcagacgcggcggccctcgagcacgacaaggcctacgaccagcagctcaaggccggagacaacccgtacctcaagtacaaccacgccgacgccgagttccaggagcggctcaaagaagatacgtcttttgggggcaacctcgggcgagcagtcttccagaccaagaagagggttctcgaaccttttggtctggttgaggaaggtgctaagacggctcctggaaagaaacgtccggtagagcagtcgccacaagagccagactcctcctcgggcattgtcaagacaggccagcagcccgctaaaaagagactcaattttggtcagactggcgacacagagtcagtccccgacccacaacctctcggagaacctccagcaaccccctcaggtgtgggatctcttacaatggcttcaggcggtggcgcaccaatggcagacaataacgaaggcgccgacggagtgggtaatgcctcaggaaattggcattgcgattccacatggctgggcgacagagtcatcaccaccagcacccgaacctgggccctgcccacctacaacaaccacctctacaagcaaatctccaacgggacatcgggaggagccaccaacgacaacgcctacttcggctacagcaccccctgggggtattttgactttaacagattccactgccacttttcaccacgtgactggcagcgactcatcaacaacaactggggattccggcctaagcgactcaacttcaagctcttcaacattcaggtcaaagaggttacggacaacaatggagtcaagaccatcgccaataaccttaccagcacggtccaggtcttcacggactcagactatcagctcccgtacgtgctcgggtcggctcacgagggctgcctcccgccgttcccagcggacgttttcatgattcctcagtacgggtatctgacgcttaatgatggaagccaggccgtgggtcgttcgtccttttactgcctggaatatttcccgtcgcaaatgctaagaacgggtaacaacttccagttcagctacgagtttgagaacgtacctttccatagcagctacgctcacagccaaagcctggaccgactaatgaatccactcatcgaccaatacttgtactatctctcaaagactattaacggttctggacagaatcaacaaacgctaaaattcagtgtggccggacccagcaacatggctgtccagggaagaaactacatacctggacccagctaccgacaacaacgtgtctcaaccactgtgactcaaaacaacaacagcgaatttgcttggcctggagcttcttcttgggctctcaatggacgtaatagcttgatgaatcctggacctgctatggccagccacaaagaaggagaggaccgtttctttcctttgtctggatctttaatttttggcaaacaaggaactggaagagacaacgtggatgcggacaaagtcatgataaccaacgaagaagaaattaaaactactaacccggtagcaacggagtcctatggacaagtggccacaaaccaccagggccagagtggccgcggcgatctgggcctgagcgcccaggcggcccagaccggctgggttcaaaaccaaggaatacttccgggtatggtttggcaggacagagatgtgtacctgcaaggacccatttgggccaaaattcctcacacggacggcaactttcacccttctccgctgatgggagggtttggaatgaaacacccgcctcctcagatcctcatcaaaaacacacctgtacctgcggatcctccaacggccttcaacaaggacaagctgaactctttcatcacccagtattctactggccaagtcagcgtggagatcgagtgggagctgcagaaggaaaacagcaagcgctggaacccggagatccagtacacttccaactattacaagtctaataatgttgaatttgctgttaatactgaaggtgtatatagtgaaccccgccccattggcaccagatacctgactcgtaatctgtaa

SEQ ID NO: 34 - protein, 745 aa, Artificial
  AAVH15_P1 capsid polypeptide
MAADGYLPDWLEDNLSEGIREWWDLKPGAPKPKANQQKQDDGRGLVLPGYKYLGPFNGLDKGEPVNAADAAALEHDKAYDQQLKAGDNPYLRYNHADAEFQERLQEDTSFGGNLGRAVFQAKKRVLEPFGLVEEGAKTAPGKKRPVEQSPQEPDSSSGIGKTGQQPAKKRLNFGQTGDSESVPDPQPLGEPPATPAAVGPTTMASGGGAPVADNNEGADGVGSSSGNWHCDSQWLGDRVITTSTRTWALPTYNNHLYKQISNSTSGGSSNDNAYFGYSTPWGYFDFNRFHCHFSPRDWQRLINNNWGFRPKRLNFKLFNIQVKEVTDNNGVKTIANNLTSTVQVFTDSDYQLPYVLGSAHEGCLPPFPADVFMIPQYGYLTLNDGSQAVGRSSFYCLEYFPSQMLRTGNNFQFSYEFENVPFHSSYAHSQSLDRLMNPLIDQYLYYLSKTINGSGQNQQTLKFSVAGPSNMAVQGRNYIPGPSYRQQRVSTTVTQNNNSEFAWPGASSWALNGRNSLMNPGPAMASHKEGEDRFFPLSGSLIFGKQGTGRDNVDADKVMITNEEEIKTTNPVATESYGQVATNHQGQSGRGDLGLSAQAAQTGWVQNQGILPGMVWQDRDVYLQGPIWAKIPHTDGNFHPSPLMGGFGLKHPPPQILIKNTPVPADPPAEFSATKFASFITQYSTGQVSVEIEWELQKENSKRWNPEVQYTSNYAKSANVDFTVDNNGLYTEPRPIGTRYLTRPL

SEQ ID NO: 35 - DNA, 2238 bp, Artificial
  AAVH15_P1 capsid polypeptide encoding
atggctgccgatggttatcttccagattggctcgaggacaacctctctgagggcattcgcgagtggtgggacttgaaacctggagccccgaaacccaaagccaaccagcaaaagcaggacgacggccggggtctggtgcttcctggctacaagtacctcggacccttcaacggactcgacaagggggagcccgtcaacgcggcggatgcagcggccctcgagcacgacaaggcctacgaccagcagctcaaagcgggtgacaatccgtaccttcggtataaccacgccgacgccgagtttcaggagcgtctgcaagaagatacgtcttttgggggcaacctcgggcgagcagtcttccaggccaagaagagggttctcgaaccttttggtctggttgaggaaggtgctaagacggctcctggaaagaaacgtccggtagagcagtcgccacaagagccagactcctcctcgggcattggcaagacaggccagcagcccgctaaaaagagactcaattttggtcagactggcgactcagagtcagtccccgacccacaacctctcggagaacctccagcaacccccgctgctgtgggacctactacaatggcttcaggtggtggcgcaccagtggcagacaataacgaaggtgccgatggagtgggtagttcctcgggaaattggcattgcgattcccaatggctgggggacagagtcatcaccaccagcacccgaacctgggccctgcccacctacaacaatcacctctacaagcaaatctccaacagcacatctggaggatcttcaaatgacaacgcctacttcggctacagcaccccctgggggtattttgacttcaacagattccactgccacttctcaccacgtgactggcagcgactcatcaacaacaactggggattccggcctaagcgactcaacttcaagctcttcaacattcaggtcaaagaggttacggacaacaatggagtcaagaccatcgccaataaccttaccagcacggtccaggtcttcacggactcagactatcagctcccgtacgtgctcgggtcggctcacgagggctgcctcccgccgttcccagcggacgttttcatgattcctcagtacgggtatctgacgcttaatgatggaagccaggccgtgggtcgttcgtccttttactgcctggaatatttcccgtcgcaaatgctaagaacgggtaacaacttccagttcagctacgagtttgagaacgtacctttccatagcagctacgctcacagccaaagcctggaccgactaatgaatccactcatcgaccaatacttgtactatctctcaaagactattaacggttctggacagaatcaacaaacgctaaaattcagtgtggccggacccagcaacatggctgtccagggaagaaactacatacctggacccagctaccgacaacaacgtgtctcaaccactgtgactcaaaacaacaacagcgaatttgcttggcctggagcttcttcttgggctctcaatggacgtaatagcttgatgaatcctggacctgctatggccagccacaaagaaggagaggaccgtttctttcctttgtctggatctttaatttttggcaaacaaggaactggaagagacaacgtggatgcggacaaagtcatgataaccaacgaagaagaaattaaaactactaacccggtagcaacggagtcctatggacaagtggccacaaaccaccagggccagagtggccgcggcgatctgggcctgagcgcccaggcggcccagaccggctgggttcaaaaccaaggaatacttccgggtatggtttggcaggacagagatgtgtacctgcaaggacccatttgggccaaaattcctcacacggacggcaacttccacccgtctccgctgatgggcggctttggcctgaaacatcctccgcctcagatcctgatcaagaacacgcctgtacctgcggatcctccggcagagttttcggctacaaagtttgcttcattcatcacccagtattccacaggacaagtgagcgtggagattgaatgggagctgcagaaagaaaacagcaaacgctggaatcccgaagtgcagtatacatctaactatgcaaaatctgccaacgttgatttcactgtggacaacaatggactttatactgagcctcgccccattggcacccgttacctcacccgtcccctgtaa

SEQ ID NO: 36 - protein, 6 aa, Artificial
  AAV1  insertion site 1
STDPAT

SEQ ID NO: 37 - protein, 6 aa, Artificial
  AAV1  insertion site 2
SSSTDP

SEQ ID NO: 38 - protein, 6 aa, Artificial
  AAV2  insertion site 1
GNRQAA

SEQ ID NO: 39 - protein, 6 aa, Artificial
  AAV2  insertion site 2
RGNRQA

SEQ ID NO: 40 - protein, 6 aa, Artificial
  AAV3b  insertion site 1
LQSSNT

SEQ ID NO: 41 - protein, 6 aa, Artificial
  AAV3b  insertion site 2
SSNTAP

SEQ ID NO: 42 - protein, 6 aa, Artificial
  AAV4  insertion site 1
DQSNSN

SEQ ID NO: 43 - protein, 6 aa, Artificial
  AAV4  insertion site 2
SNSNLP

SEQ ID NO: 44 - protein, 6 aa, Artificial
  AAV5  insertion site 1
NQSSTT

SEQ ID NO: 45 - protein, 6 aa, Artificial
  AAV5  insertion site 2
SSTTAP

SEQ ID NO: 46 - protein, 6 aa, Artificial
  AAV6  insertion site 1
STDPAT

SEQ ID NO: 47 - protein, 6 aa, Artificial
  AAV6  insertion site 2
SSSTDP

SEQ ID NO: 48 - protein, 6 aa, Artificial
  AAV7  insertion site 1
AANTAA

SEQ ID NO: 49 - protein, 6 aa, Artificial
  AAV8  insertion site 1
QQNTAP

SEQ ID NO: 50 - protein, 6 aa, Artificial
  AAV9 insertion site 1
SAQAQA

SEQ ID NO: 51 - protein, 6 aa, Artificial
  AAVrh10  insertion site 1
QQNAAP

SEQ ID NO: 52 - protein, 6 aa, Artificial
  AAVpo.1  insertion site 1
NQNSNT

SEQ ID NO: 53 - protein, 6 aa, Artificial
  AAVpo.1  insertion site 2
NSNTHP

SEQ ID NO: 54 - protein, 6 aa, Artificial
  AAV12 insertion site 1
NQNATT

SEQ ID NO: 55 - protein, 6 aa, Artificial
  AAV12 insertion site 2
NATTAP